European Patent Application EP 4 722 248 A1, published April 8, 2026. Title: Bispecific antibody that recognizes CCR8 as antigen. Applicant: 塩野義製薬株式会社. The sequence listing filed with the application follows.

SEQUENCE LISTING (96 sequences)

SEQ ID NO: 1 - protein, 21 aa, Homo sapiens
MALPVTALLLPLALLLHAARP

SEQ ID NO: 2 - protein, 15 aa, synthetic construct
GGGGSGGGGSGGGGS

SEQ ID NO: 3 - protein, 9 aa, synthetic construct
ANASGGGGS

SEQ ID NO: 4 - protein, 4 aa, synthetic construct
ANAS

SEQ ID NO: 5 - protein, 26 aa, synthetic construct
ANAEPPPPLPPPPEPPPPDASGGGGS

SEQ ID NO: 6 - protein, 111 aa, synthetic construct
ANAEPPPPLPPPPEPPPPDAEPPPPLPPPPEPPPPDAEPPPPLPPPPEPPPPDAEPPPPLPPPPEPPPPDAEPPPPLPPPPEPPPPDAEPPPPLPPPPEPPPPDASGGGGS

SEQ ID NO: 7 - protein, 243 aa, synthetic construct
DIKLQQSGAELARPGASVKMSCKTSGYTFTRYTMHWVKQRPGQGLEWIGYINPSRGYTNYNQKFKDKATLTTDKSSSTAYMQLSSLTSEDSAVYYCARYYDDHYCLDYWGQGTTLTVSSVEGGSGGSGGSGGSGGVDDIQLTQSPAIMSASPGEKVTMTCRASSSVSYMNWYQQKSGTSPKRWIYDTSKVASGVPYRFSGSGSGTSYSLTISSMEAEDAATYYCQQWSSNPLTFGAGTKLELK

SEQ ID NO: 8 - protein, 249 aa, synthetic construct
EVQLVESGGGLVQPGGSLKLSCAASGFTFNKYAMNWVRQAPGKGLEWVARIRSKYNNYATYYADSVKDRFTISRDDSKNTAYLQMNNLKTEDTAVYYCVRHGNFGNSYISYWAYWGQGTLVTVSSGGGGSGGGGSGGGGSQTVVTQEPSLTVSPGGTVTLTCGSSTGAVTSGNYPNWVQQKPGQAPRGLIGGTKFLAPGTPARFSGSLLGGKAALTLSGVQPEDEAEYYCVLWYSNRWVFGGGTKLTVL

SEQ ID NO: 9 - protein, 254 aa, synthetic construct
EVQLVESGGGLVQPGGSLRLSCAASGFTFSTYAMNWVRQAPGKGLEWVGRIRSKYNNYATYYADSVKGRFTISRDDSKNTLYLQMNSLRAEDTAVYYCVRHGNFGDSYVSWFAYWGQGTLVTVSSGKPGSGKPGSGKPGSGKPGSQAVVTQEPSLTVSPGGTVTLTCGSSTGAVTTSNYANWVQQKPGKSPRGLIGGTNKRAPGVPARFSGSLLGGKAALTISGAQPEDEADYYCALWYSNHWVFGGGTKLTVL

SEQ ID NO: 10 - protein, 106 aa, synthetic construct
DIQLTQSPAIMSASPGEKVTMTCRASSSVSYMNWYQQKSGTSPKRWIYDTSKVASGVPYRFSGSGSGTSYSLTISSMEAEDAATYYCQQWSSNPLTFGAGTKLELK

SEQ ID NO: 11 - protein, 119 aa, synthetic construct
DIKLQQSGAELARPGASVKMSCKTSGYTFTRYTMHWVKQRPGQGLEWIGYINPSRGYTNYNQKFKDKATLTTDKSSSTAYMQLSSLTSEDSAVYYCARYYDDHYCLDYWGQGTTLTVSS

SEQ ID NO: 12 - protein, 109 aa, synthetic construct
QTVVTQEPSLTVSPGGTVTLTCGSSTGAVTSGNYPNWVQQKPGQAPRGLIGGTKFLAPGTPARFSGSLLGGKAALTLSGVQPEDEAEYYCVLWYSNRWVFGGGTKLTVL

SEQ ID NO: 13 - protein, 125 aa, synthetic construct
EVQLVESGGGLVQPGGSLKLSCAASGFTFNKYAMNWVRQAPGKGLEWVARIRSKYNNYATYYADSVKDRFTISRDDSKNTAYLQMNNLKTEDTAVYYCVRHGNFGNSYISYWAYWGQGTLVTVSS

SEQ ID NO: 14 - protein, 109 aa, synthetic construct
QAVVTQEPSLTVSPGGTVTLTCGSSTGAVTTSNYANWVQQKPGKSPRGLIGGTNKRAPGVPARFSGSLLGGKAALTISGAQPEDEADYYCALWYSNHWVFGGGTKLTVL

SEQ ID NO: 15 - protein, 125 aa, synthetic construct
EVQLVESGGGLVQPGGSLRLSCAASGFTFSTYAMNWVRQAPGKGLEWVGRIRSKYNNYATYYADSVKGRFTISRDDSKNTLYLQMNSLRAEDTAVYYCVRHGNFGDSYVSWFAYWGQGTLVTVSS

SEQ ID NO: 16 - protein, 10 aa, synthetic construct
RASSSVSYMN

SEQ ID NO: 17 - protein, 7 aa, synthetic construct
DTSKVAS

SEQ ID NO: 18 - protein, 9 aa, synthetic construct
QQWSSNPLT

SEQ ID NO: 19 - protein, 5 aa, synthetic construct
RYTMH

SEQ ID NO: 20 - protein, 17 aa, synthetic construct
YINPSRGYTNYNQKFKD

SEQ ID NO: 21 - protein, 10 aa, synthetic construct
YYDDHYCLDY

SEQ ID NO: 22 - protein, 14 aa, synthetic construct
GSSTGAVTSGNYPN

SEQ ID NO: 23 - protein, 7 aa, synthetic construct
GTKFLAP

SEQ ID NO: 24 - protein, 9 aa, synthetic construct
VLWYSNRWV

SEQ ID NO: 25 - protein, 5 aa, synthetic construct
KYAMN

SEQ ID NO: 26 - protein, 19 aa, synthetic construct
RIRSKYNNYATYYADSVKD

SEQ ID NO: 27 - protein, 14 aa, synthetic construct
HGNFGNSYISYWAY

SEQ ID NO: 28 - protein, 14 aa, synthetic construct
GSSTGAVTTSNYAN

SEQ ID NO: 29 - protein, 7 aa, synthetic construct
GTNKRAP

SEQ ID NO: 30 - protein, 9 aa, synthetic construct
ALWYSNHWV

SEQ ID NO: 31 - protein, 5 aa, synthetic construct
TYAMN

SEQ ID NO: 32 - protein, 19 aa, synthetic construct
RIRSKYNNYATYYADSVKG

SEQ ID NO: 33 - protein, 14 aa, synthetic construct
HGNFGDSYVSWFAY

SEQ ID NO: 34 - protein, 122 aa, synthetic construct
QVQLVESGGGLVQPGGSLRLSCAASGLTFSSYNMGWFRQAPGQGLEAVASITWSGRDTFYADSVKGRFTISRDNSKNTLYLQMNSLRAEDTAVYYCAANPWPVAAPRSGTYWGQGTLVTVSS

SEQ ID NO: 35 - protein, 5 aa, synthetic construct
SYNMG

SEQ ID NO: 36 - protein, 17 aa, synthetic construct
SITWSGRDTFYADSVKG

SEQ ID NO: 37 - protein, 13 aa, synthetic construct
NPWPVAAPRSGTY

SEQ ID NO: 38 - protein, 6 aa, synthetic construct
HHHHHH

SEQ ID NO: 39 - protein, 250 aa, synthetic construct
EVQLVESGGALVKPGGSLRLSCAASGFTFSTYAMYWVRQAPGKGLEWVGRIRSKSNNYATYYADSVKDRFTISRDDSKNTLYLQMNSLKTEDTAVYYCTRGGYGNYRYAMDYWGQGTTVTVSSGGGGSGGGGSGGGGSEIVLTQSPGTLSLSPGERATLSCRSSKSLLHSNGNTYLYWYQQKPGQAPRLLIYRVSNLASGIPDRFSGSGSGTDFTLTISRLEPEDFAVYYCMQHLEYPFTFGQGTKLEIK

SEQ ID NO: 40 - protein, 250 aa, synthetic construct
EVQLVETGGGLVQPKGSLKLSCAASGFTFNTNAMNWVRQAPGKGLEWVARIRSKSNNYATYYADSVKDRFTISRDDSQSMLYLQMNNLKTEDTAMYYCVREIRPLGDFDVWGAGTTVTVSSGGGGSGGGGSGGGGSDIVMTQAAPSVPVTPGESVSISCRSSKSLLHSNGNTYLYWFLQRPGQSPQLLIYRMSNLASGVPDRFSGSGSGTAFTLRISRVEAEDVGVYYCMQHLEYPFTFGSGTKLEIKRA

SEQ ID NO: 41 - protein, 251 aa, synthetic construct
EVQLVETGGGLVQPKGSLKLSCAASGFTFNTNAMNWVRQTPGKGLEWVARIRSKSNNYATYYADSVKDRFTISRDDSQSMLYLQMNNLKTEDTAVYYCVREIRPLGDFDVWGAGTTVTVSSGGGGSGGGGSGGGGSEIVMTQAVPSVPVTPGESVSISCRSSKSLLHSNGNTYLYWFLQRPGQSPQLLIYRMSNLASGVPDRFSGSGSGTAFTLRISRVEAEDVGVYYCMQHLEYPFTFGSGTKLEIKRAD

SEQ ID NO: 42 - protein, 245 aa, synthetic construct
QVQLKQSGPSLVQPSQSLSITCTVSGFSLTAYGVHWIRQSPGKGQEWLGVIWRGGSTDYNAAFMSRLTITKDNSKSQVFFKMNSLQADDTAIYYCAKKGGSYAMDYWGQGTSVTVSSGGGGSGGGGSGGGGSDVVLTQTPLSLPVSLGGQASISCRSSQSLVHSNGNTYLHWYLQKPGQSPKLLIYKVSNRFSGVPDRFSGSGSGTDFTLKISRVEAEDLGVYFCSQSTQVPLTFGAGTKLELKR

SEQ ID NO: 43 - protein, 251 aa, synthetic construct
EVQVLESGGGLVQPGNSLKLSCATSGFTFSTAWMYWYRQFPEKRLEWVARIKAKSNNYGTDYTESVKGRFTISRDDSKSSIYLQMNNLKEEDTAIYYCALYYYSSSHWFAYWGQGTLVTVSSGGGGSGGGGSGGGGSDVVLTQTPVAQPVTLGDQASISCRSSQSLVHSSGNTYLEWYLQRPGQSPQLLIYKVSNRFSGVPDRFIGSGSGSDFTLKISRVEPEDLGVYYCFQATHVPWTFGGGTKLELKRA

SEQ ID NO: 44 - protein, 250 aa, synthetic construct
EVQLVESDGGLVQPGRSLKLSCAASGFTFSDYYMAWVRQAPTKGLEWVATITYDVYSTYYRDSVKGRFTISRDNAKSTLYLQMDSLRSEDTATYYCARHGGDGYNSGNWFAYWGQGTLVTVSSGGGGSGGGGSGGGGSDIVLTQSPALAVSLGQRATISCRASQSVSISRYNIMHWYQQKPGQQPKLLIYRASNLASGIPARFSGSGSGTDFTLTINPVQADDIATYYCQQSRESPPTFGGGTKLELKRA

SEQ ID NO: 45 - protein, 112 aa, synthetic construct
EIVLTQSPGTLSLSPGERATLSCRSSKSLLHSNGNTYLYWYQQKPGQAPRLLIYRVSNLASGIPDRFSGSGSGTDFTLTISRLEPEDFAVYYCMQHLEYPFTFGQGTKLEIK

SEQ ID NO: 46 - protein, 123 aa, synthetic construct
EVQLVESGGALVKPGGSLRLSCAASGFTFSTYAMYWVRQAPGKGLEWVGRIRSKSNNYATYYADSVKDRFTISRDDSKNTLYLQMNSLKTEDTAVYYCTRGGYGNYRYAMDYWGQGTTVTVSS

SEQ ID NO: 47 - protein, 114 aa, synthetic construct
DIVMTQAAPSVPVTPGESVSISCRSSKSLLHSNGNTYLYWFLQRPGQSPQLLIYRMSNLASGVPDRFSGSGSGTAFTLRISRVEAEDVGVYYCMQHLEYPFTFGSGTKLEIKRA

SEQ ID NO: 48 - protein, 121 aa, synthetic construct
EVQLVETGGGLVQPKGSLKLSCAASGFTFNTNAMNWVRQAPGKGLEWVARIRSKSNNYATYYADSVKDRFTISRDDSQSMLYLQMNNLKTEDTAMYYCVREIRPLGDFDVWGAGTTVTVSS

SEQ ID NO: 49 - protein, 115 aa, synthetic construct
EIVMTQAVPSVPVTPGESVSISCRSSKSLLHSNGNTYLYWFLQRPGQSPQLLIYRMSNLASGVPDRFSGSGSGTAFTLRISRVEAEDVGVYYCMQHLEYPFTFGSGTKLEIKRAD

SEQ ID NO: 50 - protein, 121 aa, synthetic construct
EVQLVETGGGLVQPKGSLKLSCAASGFTFNTNAMNWVRQTPGKGLEWVARIRSKSNNYATYYADSVKDRFTISRDDSQSMLYLQMNNLKTEDTAVYYCVREIRPLGDFDVWGAGTTVTVSS

SEQ ID NO: 51 - protein, 113 aa, synthetic construct
DVVLTQTPLSLPVSLGGQASISCRSSQSLVHSNGNTYLHWYLQKPGQSPKLLIYKVSNRFSGVPDRFSGSGSGTDFTLKISRVEAEDLGVYFCSQSTQVPLTFGAGTKLELKR

SEQ ID NO: 52 - protein, 117 aa, synthetic construct
QVQLKQSGPSLVQPSQSLSITCTVSGFSLTAYGVHWIRQSPGKGQEWLGVIWRGGSTDYNAAFMSRLTITKDNSKSQVFFKMNSLQADDTAIYYCAKKGGSYAMDYWGQGTSVTVSS

SEQ ID NO: 53 - protein, 114 aa, synthetic construct
DVVLTQTPVAQPVTLGDQASISCRSSQSLVHSSGNTYLEWYLQRPGQSPQLLIYKVSNRFSGVPDRFIGSGSGSDFTLKISRVEPEDLGVYYCFQATHVPWTFGGGTKLELKRA

SEQ ID NO: 54 - protein, 122 aa, synthetic construct
EVQVLESGGGLVQPGNSLKLSCATSGFTFSTAWMYWYRQFPEKRLEWVARIKAKSNNYGTDYTESVKGRFTISRDDSKSSIYLQMNNLKEEDTAIYYCALYYYSSSHWFAYWGQGTLVTVSS

SEQ ID NO: 55 - protein, 112 aa, synthetic construct
DIVLTQSPALAVSLGQRATISCRASQSVSISRYNIMHWYQQKPGQQPKLLIYRASNLASGIPARFSGSGSGTDFTLTINPVQADDIATYYCQQSRESPPTFGGGTKLELKRA

SEQ ID NO: 56 - protein, 123 aa, synthetic construct
EVQLVESDGGLVQPGRSLKLSCAASGFTFSDYYMAWVRQAPTKGLEWVATITYDVYSTYYRDSVKGRFTISRDNAKSTLYLQMDSLRSEDTATYYCARHGGDGYNSGNWFAYWGQGTLVTVSS

SEQ ID NO: 57 - protein, 16 aa, synthetic construct
RSSKSLLHSNGNTYLY

SEQ ID NO: 58 - protein, 7 aa, synthetic construct
RVSNLAS

SEQ ID NO: 59 - protein, 9 aa, synthetic construct
MQHLEYPFT

SEQ ID NO: 60 - protein, 5 aa, synthetic construct
TYAMY

SEQ ID NO: 61 - protein, 19 aa, synthetic construct
RIRSKSNNYATYYADSVKD

SEQ ID NO: 62 - protein, 12 aa, synthetic construct
GGYGNYRYAMDY

SEQ ID NO: 63 - protein, 7 aa, synthetic construct
RMSNLAS

SEQ ID NO: 64 - protein, 5 aa, synthetic construct
TNAMN

SEQ ID NO: 65 - protein, 10 aa, synthetic construct
EIRPLGDFDV

SEQ ID NO: 66 - protein, 16 aa, synthetic construct
RSSQSLVHSNGNTYLH

SEQ ID NO: 67 - protein, 7 aa, synthetic construct
KVSNRFS

SEQ ID NO: 68 - protein, 9 aa, synthetic construct
SQSTQVPLT

SEQ ID NO: 69 - protein, 5 aa, synthetic construct
AYGVH

SEQ ID NO: 70 - protein, 16 aa, synthetic construct
VIWRGGSTDYNAAFMS

SEQ ID NO: 71 - protein, 9 aa, synthetic construct
KGGSYAMDY

SEQ ID NO: 72 - protein, 16 aa, synthetic construct
RSSQSLVHSSGNTYLE

SEQ ID NO: 73 - protein, 9 aa, synthetic construct
FQATHVPWT

SEQ ID NO: 74 - protein, 5 aa, synthetic construct
TAWMY

SEQ ID NO: 75 - protein, 19 aa, synthetic construct
RIKAKSNNYGTDYTESVKG

SEQ ID NO: 76 - protein, 11 aa, synthetic construct
YYYSSSHWFAY

SEQ ID NO: 77 - protein, 15 aa, synthetic construct
RASQSVSISRYNIMH

SEQ ID NO: 78 - protein, 7 aa, synthetic construct
RASNLAS

SEQ ID NO: 79 - protein, 9 aa, synthetic construct
QQSRESPPT

SEQ ID NO: 80 - protein, 5 aa, synthetic construct
DYYMA

SEQ ID NO: 81 - protein, 17 aa, synthetic construct
TITYDVYSTYYRDSVKG

SEQ ID NO: 82 - protein, 14 aa, synthetic construct
HGGDGYNSGNWFAY

SEQ ID NO: 83 - protein, 355 aa, Homo sapiens
MDYTLDLSVTTVTDYYYPDIFSSPCDAELIQTNGKLLLAVFYCLLFVFSLLGNSLVILVLVVCKKLRSITDVYLLNLALSDLLFVFSFPFQTYYLLDQWVFGTVMCKVVSGFYYIGFYSSMFFITLMSVDRYLAVVHAVYALKVRTIRMGTTLCLAVWLTAIMATIPLLVFYQVASEDGVLQCYSFYNQQTLKWKIFTNFKMNILGLLIPFTIFMFCYIKILHQLKRCQNHNKTKAIRLVLIVVIASLLFWVPFNVVLFLTSLHSMHILDGCSISQQLTYATHVTEIISFTHCCVNPVIYAFVGEKFKKHLSEIFQKSCSQIFNYLGRQMPRESCEKSSSCQQHSSRSSSVDYIL

SEQ ID NO: 84 - protein, 238 aa, synthetic construct
EVQLVESGGGLVQPGKSLKLSCEASGFTFSGYGMHWVRQAPGRGLESVAYITSSSINIKYADAVKGRFTVSRDNAKNLLFLQMNILKSEDTAMYYCARFDWDKNYWGQGTMVTVSSGGGGSGGGGSGGGGSDIQMTQSPSSLPASLGDRVTINCQASQDISNYLNWYQQKPGKAPKLLIYYTNKLADGVPSRFSGSGSGRDSSFTISSLESEDIGSYYCQQYYNYPWTFGPGTKLEIK

SEQ ID NO: 85 - protein, 109 aa, synthetic construct
DIQMTQSPSSLPASLGDRVTINCQASQDISNYLNWYQQKPGKAPKLLIYYTNKLADGVPSRFSGSGSGRDSSFTISSLESEDIGSYYCQQYYNYPWTFGPGTKLEIKRA

SEQ ID NO: 86 - protein, 116 aa, synthetic construct
EVQLVESGGGLVQPGKSLKLSCEASGFTFSGYGMHWVRQAPGRGLESVAYITSSSINIKYADAVKGRFTVSRDNAKNLLFLQMNILKSEDTAMYYCARFDWDKNYWGQGTMVTVSS

SEQ ID NO: 87 - protein, 11 aa, synthetic construct
QASQDISNYLN

SEQ ID NO: 88 - protein, 7 aa, synthetic construct
YTNKLAD

SEQ ID NO: 89 - protein, 9 aa, synthetic construct
QQYYNYPWT

SEQ ID NO: 90 - protein, 5 aa, synthetic construct
GYGMH

SEQ ID NO: 91 - protein, 17 aa, synthetic construct
YITSSSINIKYADAVKG

SEQ ID NO: 92 - protein, 7 aa, synthetic construct
FDWDKNY

SEQ ID NO: 93 - protein, 24 aa, synthetic construct
ANASGGGGSGGGGSGGGGSGGGGS

SEQ ID NO: 94 - protein, 6 aa, synthetic construct
GSGGGG

SEQ ID NO: 95 - protein, 484 aa, synthetic construct
DKTHTCPPCPAPELLGGPSVFLFPPKPKDTLMISRTPEVTCVVVDVSHEDPEVKFNWYVDGVEVHNAKTKPCEEQYGSTYRCVSVLTVLHQDWLNGKEYKCKVSNKALPAPIEKTISKAKGQPREPQVYTLPPSREEMTKNQVSLTCLVKGFYPSDIAVEWESNGQPENNYKTTPPVLDSDGSFFLYSKLTVDKSRWQQGNVFSCSVMHEALHNHYTQKSLSLSPGKGGGGSGGGGSGGGGSGGGGSGGGGSGGGGSDKTHTCPPCPAPELLGGPSVFLFPPKPKDTLMISRTPEVTCVVVDVSHEDPEVKFNWYVDGVEVHNAKTKPCEEQYGSTYRCVSVLTVLHQDWLNGKEYKCKVSNKALPAPIEKTISKAKGQPREPQVYTLPPSREEMTKNQVSLTCLVKGFYPSDIAVEWESNGQPENNYKTTPPVLDSDGSFFLYSKLTVDKSRWQQGNVFSCSVMHEALHNHYTQKSLSLSPGK

SEQ ID NO: 96 - protein, 520 aa, synthetic construct
MDMRVPAQLLGLLLLWLRGARCEVQLVESGGGLVKPGGSLRLSCAASGFTFSNARMGWVRQAPGKGLEWVGRIKSKTEGGTRDYAAPVKGRFTISRDDSKNTLYLQMNSLKTEDTAVYYCTSYSGVWGQGTMVTVSSGGGGSGGGGSGGGGSDIVMTQSPDSLAVSLGERATINCKSSQSVLYSSNNKNYLAWYHQKPGQSPKLLISWASTRESGVPDRFSGSGSGTDFTLTINSLQAEDVAVYYCQQYYSIPITFGGGTKVEIKRGGGGSEVQLVESGGGLVQPGGSLKLSCAASGFTFNKYAINWVRQAPGKGLEWVARIRSKYNNYADAVKDRFTISRDDSKNTVYLQMNNLKTEDTAVCARAGNFGSSYISYWAYWGQGTLVTVSSGGGGSGGGGSGGGGSQTVVTQEPSLTVSPGGTVTITCGSSTGAVTSGNYPNWVQKKPGQAPRGLIGGTKFLAPGTPARFSGSLSGGKAALTLSGVQPEDEAEYYCVLWYSNRWVFGSGTKLTVLHHHHHH